European Patent Application EP 4 356 727 A2, published April 24, 2024. Title: Compositions and methods for the treatment of dominantly-inherited catecholaminergic polymorphic ventricular tachycardia. Applicant: Istituti Clinici Scientifici Maugeri S.p.A. S.B. The sequence listing filed with the application follows.

SEQUENCE LISTING (7 sequences)

SEQ ID NO: 1 - protein, 399 aa, Homo sapiens
  source 1..399: note = Wild-type human CASQ2 protein
MKRTHLFIVGIYFLSSCRAEEGLNFPTYDGKDRVVSLSEKNFKQVLKKYDLLCLYYHEPVSSDKVTQKQFQLKEIVLELVAQVLEHKAIGFVMVDAKKEAKLAKKLGFDEEGSLYILKGDRTIEFDGEFAADVLVEFLLDLIEDPVEIISSKLEVQAFERIEDYIKLIGFFKSEDSEYYKAFEEAAEHFQPYIKFFATFDKGVAKKLSLKMNEVDFYEPFMDEPIAIPNKPYTEEELVEFVKEHQRPTLRRLRPEEMFETWEDDLNGIHIVAFAEKSDPDGYEFLEILKQVARDNTDNPDLSILWIDPDDFPLLVAYWEKTFKIDLFRPQIGVVNVTDADSVWMEIPDDDDLPTAEELEDWIEDVLSGKINTEDDDEDDDDDDNSDEEDNDDSDDDDDE

SEQ ID NO: 2 - DNA, 1200 bp, Homo sapiens
  source 1..1200: mol_type = other DNA; note = Wild-type human CASQ2 cDNA
atgaagagaactcacttgtttattgtggggatttattttctgtcctcttgcagggcagaagaggggcttaatttccccacatatgatgggaaggaccgagtggtaagtctttccgagaagaacttcaagcaggttttaaagaaatatgacttgctttgcctctactaccatgagccggtgtcttcagataaggtcacgcaaaaacagttccaactgaaagaaatcgtgcttgagcttgtggcccaggtccttgaacataaagctataggctttgtgatggtggatgccaagaaagaagccaagcttgccaagaaactgggttttgatgaagaaggaagcctgtatattcttaagggtgatcgcacaatagagtttgatggcgagtttgcagctgatgtcttggtggagttcctcttggatctaattgaagacccagtggagatcatcagcagcaaactggaagtccaagccttcgaacgcattgaagactacatcaaactcattggctttttcaagagtgaggactcagaatactacaaggcttttgaagaagcagctgaacacttccagccttacatcaaattctttgccacctttgacaaaggggttgcaaagaaattatctttgaagatgaatgaggttgacttctatgagccatttatggatgagcccattgccatccccaacaaaccttacacagaagaggagctggtggagtttgtgaaggaacaccaaagacccactctacgtcgcctgcgcccagaagaaatgtttgaaacatgggaagatgatttgaatgggatccacattgtggcctttgcagagaagagtgatccagatggctacgaattcctggagatcctgaaacaggttgcccgggacaatactgacaaccccgatctgagcatcctgtggatcgacccggacgactttcctctgctcgttgcctactgggagaagactttcaagattgacctattcaggccacagattggggtggtgaatgtcacagatgctgacagtgtctggatggagattccagatgatgacgatcttccaactgctgaggagctggaggactggattgaggatgtgctttctggaaagataaacactgaagatgatgatgaagatgatgatgatgatgataattctgatgaagaggataatgatgacagtgatgacgatgatgatgaatag

SEQ ID NO: 3 - protein, 415 aa, Mus musculus
  source 1..415: note = Wild-type murine CASQ2 protein
MKRIYLLMVGVYLLSLSGAEEGLNFPTYDGKDRVVSLSEKNLKQMLKRYDLLCLYYHEPVSSDKVSQKQFQLKEIVLELVAQVLEHKNIGFVMVDSRKEAKLAKRLGFSEEGSLYVLKGDRTIEFDGEFAADVLVEFLLDLIEDPVEIVNNKLEVQAFERIEDQTKLLGFFKNEDSEYYKAFQEAAEHFQPYIKFFATFDKAVAKKLSLKMNEVGFYEPFMDEPNVIPNKPYTEEELVEFVKEHQRPTLRRLRPEDMFETWEDDLNGIHIVAFAEKSDPDGYEFLEILKQVARDNTDNPDLSILWIDPDDFPLLVAYWEKTFKIDLFKPQIGVVNVTDADSIWMEIPDDDDLPTAEELEDWIEDVLSGKINTEDDDNEDEDDDGDDNDDDDDDDDDNDNSDEDNEDSDDDDDDDE

SEQ ID NO: 4 - DNA, 1248 bp, Mus musculus
  source 1..1248: mol_type = other DNA; note = Wild-type murine CASQ2 cDNA
atgaagaggatttacctgctcatggtgggggtttatctgctgtccctgagcggggcagaagaggggctgaacttccccacgtacgatgggaaagaccgagtggtcagcctttctgagaagaacctcaagcagatgttgaagagatatgatttgctctgtctctattaccacgaacctgtgtcttcagacaaggtctcacaaaaacagttccagctgaaggagattgtactggagcttgtggcccaggtcctggaacataaaaacataggctttgtgatggtggattcgaggaaagaggccaagcttgctaagaggctgggattcagtgaagaaggaagcctgtatgttctgaagggtgaccgcacgattgagtttgacggggagttcgcagcagatgtcttagtggaatttctcttggatctcattgaagacccagtggagatcgtgaataacaagctggaggtccaggcctttgagcgcatcgaggaccagaccaagctccttggcttcttcaagaatgaggactcagaatattacaaagcattccaagaggcagctgaacacttccagccttacatcaagttctttgccacctttgacaaggcggtggcaaagaagttatccttgaagatgaacgaagttggcttctatgagccatttatggatgagcccaacgtcatccctaacaaaccgtacacagaagaggagcttgtggagtttgtgaaggaacatcaaagacccaccctacgtcgcttgcgcccagaggacatgtttgaaacatgggaagacgacttgaatgggatccacatcgtggcctttgcggagaagagtgacccagatggctatgagttcctagagatcctgaaacaggttgcccgggacaacactgacaatcctgacttgagcatcttgtggattgacccagatgactttccactgcttgttgcttactgggagaagactttcaagattgacctgttcaagccacagattggggtggtgaatgtaaccgatgctgacagtatctggatggagatcccagatgatgacgacctgcccacagctgaggagctggaagactggattgaagatgtgctttctggaaagatcaacactgaagatgatgacaatgaagatgaagatgatgatggtgatgacaacgatgacgatgatgatgacgacgatgataatgataattctgatgaggataatgaagacagtgatgatgacgatgatgacgatgaatag

SEQ ID NO: 5 - DNA, 40 bp, synthetic construct
  source 1..40: mol_type = other DNA; note = CASQ2 Forward PCR primer
cacagcggccgcacaatgaagaggatttacctgctcatgg

SEQ ID NO: 6 - DNA, 25 bp, synthetic construct
  source 1..25: mol_type = other DNA; note = CASQ2 Reverse PCR primer
cgaagcattaaccctcactaaaggg

SEQ ID NO: 7 - DNA, 18 bp, synthetic construct
  source 1..18: mol_type = other DNA; note = V4319-K4324 RYR2 duplication
gtcgaaggtgctaaaaag